European Patent Specification EP 3 494 137 B1, published July 2, 2025. Title: New anti-hCTLA4 antibodies. Applicant: Aduro Biotech Holdings, Europe B.V. The sequence listing filed with the application follows.

SEQUENCE LISTING (59 sequences)

SEQ ID NO: 1 - protein, 5 aa, Artificial Sequence
  CDR1 heavy chain
TYWMN

SEQ ID NO: 2 - protein, 17 aa, Artificial Sequence
  CDR2 heavy chain
MIHPSDSETSLNQAFKD

SEQ ID NO: 3 - protein, 11 aa, Artificial Sequence
  CDR3 heavy chain
MGRRNPYYFDY

SEQ ID NO: 4 - protein, 11 aa, Artificial Sequence
  CDR1 light chain
RPSENLYTNLA

SEQ ID NO: 5 - protein, 7 aa, Artificial Sequence
  CDR2 light chain
GATNLAD

SEQ ID NO: 6 - protein, 9 aa, Artificial Sequence
  CDR3 light chain
QHLWGTPFT

SEQ ID NO: 7 - protein, 120 aa, Artificial Sequence
  consensus heavy chain
  VARIANT (5)..(5): May be Val or Leu
  VARIANT (6)..(6): May be Gln or Glu
  VARIANT (7)..(7): May be Ser or Ala
  VARIANT (9)..(9): May be Phe or Ala
  VARIANT (10)..(10): May be Val or Glu
  VARIANT (11)..(11): May be Val or Leu
  VARIANT (12)..(12): May be Val, Ala or Lys
  VARIANT (13)..(13): May be Arg or Lys
  VARIANT (16)..(16): May be Ala, Thr or Ser
  VARIANT (20)..(20): May be Ile or Val
  VARIANT (38)..(38): May be Lys or Arg
  VARIANT (40)..(40): May be Ala or Arg
  VARIANT (43)..(43): May be Lys or Gln
  VARIANT (48)..(48): May be Ile or Met
  VARIANT (67)..(67): May be Lys or Arg
  VARIANT (68)..(68): May be Val or Ala
  VARIANT (69)..(69): May be Lys or Thr
  VARIANT (70)..(70): May be Leu, Ile or Met
  VARIANT (72)..(72): May be Ala or Arg
  VARIANT (73)..(73): May be Ala or Asp
  VARIANT (74)..(74): May be Thr, Glu or Lys
  VARIANT (76)..(76): May be Thr or Ala
  VARIANT (78)..(78): May be Thr or Ile
  VARIANT (79)..(79): May be Ala or Val
  VARIANT (81)..(81): May be Leu or Met
  VARIANT (82)..(82): May be Glu or Gln
  VARIANT (83)..(83): May be Phe or Leu
  VARIANT (87)..(87): May be Arg or Thr
  VARIANT (88)..(88): May be Ser or Asn
  VARIANT (91)..(91): May be Ser or Thr
  VARIANT (99)..(99): May be Met or Ile
  VARIANT (115)..(115): May be Leu or Thr
EVQLXXXGXXXXXPGXSVKXSCKASGYSFTTYWMNWVXQXPGXGLEWXGMIHPSDSETSLNQAFKDXXXXTXXXSXSXXYXXXSSLXXEDXAVYYCARXGRRNPYYFDYWGQGTXVTVSS

SEQ ID NO: 8 - protein, 107 aa, Artificial Sequence
  consensus light chain
  VARIANT (7)..(7): May be Ser or Ala
  VARIANT (18)..(18): May be Arg or Thr
  VARIANT (48)..(48): May be Leu or Ile
  VARIANT (70)..(70): May be Asp or Glu
  VARIANT (71)..(71): May be Tyr or Phe
  VARIANT (72)..(72): May be Thr or Ser
  VARIANT (74)..(74): May be Thr or Ser
  VARIANT (80)..(80): May be Pro, Ala or Ser
  VARIANT (100)..(100): May be Gly or Gln
  VARIANT (104)..(104): May be Leu or Val
DIQMTQXPSSLSASVGDXVTITCRPSENLYTNLAWYQQKPGKAPKLLXYGATNLADGVPSRFSGSGSGTXXXLXISSLQXEDFATYYCQHLWGTPFTFGXGTKXEIK

SEQ ID NO: 9 - DNA, 360 bp, Artificial Sequence
  hCTLA4.27VH1
  CDS (1)..(360)
gaggtgcagctgctgcagtctggcgctgtgctggccagacctggcaccagcgtgaagatcagctgcaaggccagcggctacagcttcaccacctactggatgaactgggtcaagcagcggccaggccagggcctggaatggatcggaatgatccaccccagcgacagcgagacaagcctgaaccaggccttcaaggacaaggccaagctgaccgccgccacctctgcctctatcgcctacctggaattttccagcctgaccaacgaggacagcgccgtgtactactgcgcccggatgggcagacggaacccctactacttcgactactggggccagggcaccctcgtgacagtgtctagc

SEQ ID NO: 10 - protein, 120 aa, Artificial Sequence
  Synthetic Construct
EVQLLQSGAVLARPGTSVKISCKASGYSFTTYWMNWVKQRPGQGLEWIGMIHPSDSETSLNQAFKDKAKLTAATSASIAYLEFSSLTNEDSAVYYCARMGRRNPYYFDYWGQGTLVTVSS

SEQ ID NO: 11 - DNA, 360 bp, Artificial Sequence
  hCTLA4.27VH2
  CDS (1)..(360)
gaggtgcagctggtgcagtctggcgctgtgctcgtgaaacctggcgcctccgtgaaggtgtcctgcaaggccagcggctacagcttcaccacctactggatgaactgggtgcgccagaggcctggcaagggcctggaatggatcggcatgatccaccccagcgacagcgagacaagcctgaaccaggccttcaaggacaaagtgaccatcaccgccgacgagagcaccagcaccgcctacatgcagctgagcagcctgagaagcgaggacaccgccgtgtactactgcgcccggatgggcagacggaacccctactacttcgactactggggccagggcaccaccgtgacagtgtctagc

SEQ ID NO: 12 - protein, 120 aa, Artificial Sequence
  Synthetic Construct
EVQLVQSGAVLVKPGASVKVSCKASGYSFTTYWMNWVRQRPGKGLEWIGMIHPSDSETSLNQAFKDKVTITADESTSTAYMQLSSLRSEDTAVYYCARMGRRNPYYFDYWGQGTTVTVSS

SEQ ID NO: 13 - DNA, 360 bp, Artificial Sequence
  hCTLA4.27VH3
  CDS (1)..(360)
gaggtgcagctggtgcagtctggcgccgtggtggccaagcctggcagcagcgtgaaggtgtcctgtaaagccagcggctacagcttcaccacctactggatgaactgggtgcgccaggcccctggacagggcctggaatggatgggcatgatccaccccagcgacagcgagacaagcctgaaccaggccttcaaggacagagtgaccatcaccgccgacaagagcaccagcaccgcctacatggaactgagcagcctgaccagcgaggacaccgccgtgtactactgcgcccggatgggcagacggaacccctactacttcgactactggggccagggcaccaccgtgacagtgtctagc

SEQ ID NO: 14 - protein, 120 aa, Artificial Sequence
  Synthetic Construct
EVQLVQSGAVVAKPGSSVKVSCKASGYSFTTYWMNWVRQAPGQGLEWMGMIHPSDSETSLNQAFKDRVTITADKSTSTAYMELSSLTSEDTAVYYCARMGRRNPYYFDYWGQGTTVTVSS

SEQ ID NO: 15 - DNA, 360 bp, Artificial Sequence
  hCTLA4.27VH4
  CDS (1)..(360)
gaggtgcagctggtgcagtctggcgccgaagtgaagaaaccaggcgccagcgtgaaggtgtcctgcaaggccagcggctacagcttcaccacctactggatgaactgggtgcgccaggcccctggacagggcctggaatggatgggcatgatccaccccagcgacagcgagacaagcctgaaccaggccttcaaggacagagtgaccatgacccgggacaccagcacctccaccgtgtacatggaactgagcagcctgcggagcgaggacaccgccgtgtactactgcgcccggatgggcagacggaacccctactacttcgactactggggccagggcaccctcgtgacagtgtctagc

SEQ ID NO: 16 - protein, 120 aa, Artificial Sequence
  Synthetic Construct
EVQLVQSGAEVKKPGASVKVSCKASGYSFTTYWMNWVRQAPGQGLEWMGMIHPSDSETSLNQAFKDRVTMTRDTSTSTVYMELSSLRSEDTAVYYCARMGRRNPYYFDYWGQGTLVTVSS

SEQ ID NO: 17 - DNA, 360 bp, Artificial Sequence
  hCTLA4.27VH5
  CDS (1)..(360)
gaggtgcagctgctgcaggctggcgctgtgctggctagacctggcaccagcgtgaagatcagctgcaaggccagcggctacagcttcaccacctactggatgaactgggtcaagcagaggcccggcaagggcctggaatggatcggcatgatccaccccagcgacagcgagacaagcctgaaccaggccttcaaggacaaggccaagctgaccgccgccacctctgcctctatcgcctacctggaattttccagcctgaccaacgaggacagcgccgtgtactactgcgcccggatcggcagacggaacccctactacttcgactactggggccagggcaccctcgtgacagtgtctagc

SEQ ID NO: 18 - protein, 120 aa, Artificial Sequence
  Synthetic Construct
EVQLLQAGAVLARPGTSVKISCKASGYSFTTYWMNWVKQRPGKGLEWIGMIHPSDSETSLNQAFKDKAKLTAATSASIAYLEFSSLTNEDSAVYYCARIGRRNPYYFDYWGQGTLVTVSS

SEQ ID NO: 19 - DNA, 360 bp, Artificial Sequence
  hCTLA4.27VH6
  CDS (1)..(360)
gaggtgcagctgctggaatctggccctgaactcgtgcggcctggcagcagcgtgaagatcagctgtaaagccagcggctacagcttcaccacctactggatgaactgggtcaagcagaggcccggcaagggcctggaatggatcggcatgatccaccccagcgacagcgagacaagcctgaaccaggccttcaaggacaaagtgaagctgaccgccgccaccagcgcctctatcgcctacctggaattttccagcctgcggaacgaggacagcgccgtgtactactgcgcccggatgggcagacggaacccctactacttcgactactggggccagggcaccctcgtgacagtgtctagc

SEQ ID NO: 20 - protein, 120 aa, Artificial Sequence
  Synthetic Construct
EVQLLESGPELVRPGSSVKISCKASGYSFTTYWMNWVKQRPGKGLEWIGMIHPSDSETSLNQAFKDKVKLTAATSASIAYLEFSSLRNEDSAVYYCARMGRRNPYYFDYWGQGTLVTVSS

SEQ ID NO: 21 - DNA, 321 bp, Artificial Sequence
  hCTLA4.27VL1
  CDS (1)..(321)
gacatccagatgacccagagccccagcagcctgtctgccagcgtgggcgacagagtgaccatcacctgtcggcccagcgagaacctgtacaccaacctggcctggtatcagcagaagcccggcaaggcccccaaactgctgctgtacggcgccaccaatctggccgatggcgtgcccagcagattttccggctctggcagcggcaccgactacaccctgaccatctctagcctgcagcccgaggacttcgccacctactactgtcagcacctgtggggcacccccttcacctttggccagggcaccaagctggaaatcaag

SEQ ID NO: 22 - protein, 107 aa, Artificial Sequence
  Synthetic Construct
DIQMTQSPSSLSASVGDRVTITCRPSENLYTNLAWYQQKPGKAPKLLLYGATNLADGVPSRFSGSGSGTDYTLTISSLQPEDFATYYCQHLWGTPFTFGQGTKLEIK

SEQ ID NO: 23 - DNA, 321 bp, Artificial Sequence
  hCTLA4.27VL2
  CDS (1)..(321)
gacatccagatgacccagagccccagcagcctgtctgccagcgtgggcgacagagtgaccatcacctgtcggcccagcgagaacctgtacaccaacctggcctggtatcagcagaagcccggcaaggcccccaagctgctgatctacggcgccaccaatctggccgatggcgtgcccagcagattttccggctctggcagcggcaccgagttcagcctgagcatctctagcctgcagcccgaggacttcgccacctactactgtcagcacctgtggggcacccccttcacctttggcggcggaacaaaggtggaaatcaag

SEQ ID NO: 24 - protein, 107 aa, Artificial Sequence
  Synthetic Construct
DIQMTQSPSSLSASVGDRVTITCRPSENLYTNLAWYQQKPGKAPKLLIYGATNLADGVPSRFSGSGSGTEFSLSISSLQPEDFATYYCQHLWGTPFTFGGGTKVEIK

SEQ ID NO: 25 - DNA, 321 bp, Artificial Sequence
  hCTLA4.27VL3
  CDS (1)..(321)
gacatccagatgacccagagccccagcagcctgtctgccagcgtgggcgataccgtgaccatcacctgtcggcccagcgagaacctgtacaccaacctggcctggtatcagcagaagcccggcaaggcccccaaactgctgctgtacggcgccaccaatctggccgatggcgtgcccagcagattttccggctctggcagcggcaccgactacaccctgaccatctctagcctgcagagcgaggacttcgccacctactactgtcagcacctgtggggcacccccttcacctttggccagggcaccaagctggaaatcaag

SEQ ID NO: 26 - protein, 107 aa, Artificial Sequence
  Synthetic Construct
DIQMTQSPSSLSASVGDTVTITCRPSENLYTNLAWYQQKPGKAPKLLLYGATNLADGVPSRFSGSGSGTDYTLTISSLQSEDFATYYCQHLWGTPFTFGQGTKLEIK

SEQ ID NO: 27 - DNA, 321 bp, Artificial Sequence
  hCTLA4.27VL4
  CDS (1)..(321)
gacatccagatgacccagagccccagcagcctgtctgccagcgtgggcgacagagtgaccatcacctgtcggcccagcgagaacctgtacaccaacctggcctggtatcagcagaagcccggcaaggcccctaagctgctgctgtacggcgccaccaatctggccgatggcgtgcccagcagattttccggctctggcagcggcaccgactacaccctgaccatctctagcctgcagcccgaggacttcgccacctactactgccagcacctgtggggcacccccttcacatttggcggaggcaccaagctggaaatcaag

SEQ ID NO: 28 - protein, 107 aa, Artificial Sequence
  Synthetic Construct
DIQMTQSPSSLSASVGDRVTITCRPSENLYTNLAWYQQKPGKAPKLLLYGATNLADGVPSRFSGSGSGTDYTLTISSLQPEDFATYYCQHLWGTPFTFGGGTKLEIK

SEQ ID NO: 29 - DNA, 321 bp, Artificial Sequence
  hCTLA4.27VL5
  CDS (1)..(321)
gacatccagatgacccaggcccctagcagcctgtctgccagcgtgggcgacagagtgaccatcacctgtcggcccagcgagaacctgtacaccaacctggcctggtatcagcagaagcccggcaaggcccccaaactgctgctgtacggcgccaccaatctggccgatggcgtgcccagcagattttccggctctggcagcggcaccgactacaccctgacaatcagctccctgcaggccgaggacttcgccacctactactgtcagcacctgtggggcacccccttcacctttggcggcggaacaaagctggaaatcaag

SEQ ID NO: 30 - protein, 107 aa, Artificial Sequence
  Synthetic Construct
DIQMTQAPSSLSASVGDRVTITCRPSENLYTNLAWYQQKPGKAPKLLLYGATNLADGVPSRFSGSGSGTDYTLTISSLQAEDFATYYCQHLWGTPFTFGGGTKLEIK

SEQ ID NO: 31 - DNA, 360 bp, Mus musculus
  CDS (1)..(360)
caggtccaactgcagcagcctggggctgtactggtgaggcctggagtttcagtgaagctgtcctgcaaggcttctggctactccttcaccacctactggatgaactgggtgaagcagaggcctggacaaggccttgagtggattggcatgattcatccttccgatagtgaaactagtttaaatcaggcgttcaaggacaaggccacattgactatagacaaatcctccagcacagcctacatgcaactcagcagcccgacatctgaagactctgcggtctatttctgtgcaagaatgggacgtcgtaatccctattactttgactactggggccaaggcaccactctcacagtctcctca

SEQ ID NO: 32 - protein, 120 aa, Mus musculus
QVQLQQPGAVLVRPGVSVKLSCKASGYSFTTYWMNWVKQRPGQGLEWIGMIHPSDSETSLNQAFKDKATLTIDKSSSTAYMQLSSPTSEDSAVYFCARMGRRNPYYFDYWGQGTTLTVSS

SEQ ID NO: 33 - DNA, 321 bp, Mus musculus
  CDS (1)..(321)
gacatccaaatgactcagtctccagtctccctatctgtatctgtgggagaaactgtcaccatcacatgtcgaccaagtgagaatctttatactaatttagcatggtatcaacagaaacagggaaaatctcctcagctcctggtctatggtgcaacaaacctagcagatggtgtgccatcaaggttcagtggcagtggatcaggcacacagtactccctcaggatcaacagcctgcagtctgaagatttcgggacttattactgtcaacatttgtggggtactcctttcacgttcggctcggggacaaagttggaactaaaa

SEQ ID NO: 34 - protein, 107 aa, Mus musculus
DIQMTQSPVSLSVSVGETVTITCRPSENLYTNLAWYQQKQGKSPQLLVYGATNLADGVPSRFSGSGSGTQYSLRINSLQSEDFGTYYCQHLWGTPFTFGSGTKLELK

SEQ ID NO: 35 - DNA, 669 bp, Homo sapiens
  CDS (1)..(669)
atggcttgccttggatttcagcggcacaaggctcagctgaacctggctaccaggacctggccctgcactctcctgttttttcttctcttcatccctgtcttctgcaaagcaatgcacgtggcccagcctgctgtggtactggccagcagccgaggcatcgccagctttgtgtgtgagtatgcatctccaggcaaagccactgaggtccgggtgacagtgcttcggcaggctgacagccaggtgactgaagtctgtgcggcaacctacatgatggggaatgagttgaccttcctagatgattccatctgcacgggcacctccagtggaaatcaagtgaacctcactatccaaggactgagggccatggacacgggactctacatctgcaaggtggagctcatgtacccaccgccatactacctgggcataggcaacggaacccagatttatgtaattgatccagaaccgtgcccagattctgacttcctcctctggatccttgcagcagttagttcggggttgtttttttatagctttctcctcacagctgtttctttgagcaaaatgctaaagaaaagaagccctcttacaacaggggtctatgtgaaaatgcccccaacagagccagaatgtgaaaagcaatttcagccttattttattcccatcaat

SEQ ID NO: 36 - protein, 223 aa, Homo sapiens
MACLGFQRHKAQLNLATRTWPCTLLFFLLFIPVFCKAMHVAQPAVVLASSRGIASFVCEYASPGKATEVRVTVLRQADSQVTEVCAATYMMGNELTFLDDSICTGTSSGNQVNLTIQGLRAMDTGLYICKVELMYPPPYYLGIGNGTQIYVIDPEPCPDSDFLLWILAAVSSGLFFYSFLLTAVSLSKMLKKRSPLTTGVYVKMPPTEPECEKQFQPYFIPIN

SEQ ID NO: 37 - DNA, 669 bp, Artificial Sequence
  mutant CTLA4
  CDS (1)..(669)
atggcttgccttggatttcagcggcacaaggctcagctgaacctggctaccaggacctggccctgcactctcctgttttttcttctcttcatccctgtcttctgcaaagcaatgcacgtggcccagcctgctgtggtactggccagcagccgaggcatcgccagctttgtgtgtgagtatgcatctccaggcaaagccactgaggtccgggtgacagtgcttcggcaggctgacagccaggtgactgaagtctgtgcggcaacctacatgatggggaatgagttgaccttcctagatgattccatctgcacgggcacctccagtggaaatcaagtgaacctcactatccaaggactgagggccatggacacgggactctacatctgcaaggtggagctcatgtacccaccgccatactacctgggcataggcaacggaacccagatttatgtaattgatccagaaccgtgcccagattctgacttcctcctctggatccttgcagcagttagttcggggttgtttttttatagctttctcctcacagctgtttctttgagcaaaatgctaaagaaaagaagccctcttacaacaggggtcggtgtgaaaatgcccccaacagagccagaatgtgaaaagcaatttcagcctggttttattcccatcaat

SEQ ID NO: 38 - protein, 223 aa, Artificial Sequence
  Synthetic Construct
MACLGFQRHKAQLNLATRTWPCTLLFFLLFIPVFCKAMHVAQPAVVLASSRGIASFVCEYASPGKATEVRVTVLRQADSQVTEVCAATYMMGNELTFLDDSICTGTSSGNQVNLTIQGLRAMDTGLYICKVELMYPPPYYLGIGNGTQIYVIDPEPCPDSDFLLWILAAVSSGLFFYSFLLTAVSLSKMLKKRSPLTTGVGVKMPPTEPECEKQFQPGFIPIN

SEQ ID NO: 39 - DNA, 669 bp, Macaca fascicularis
  CDS (1)..(669)
atggcttgccttggatttcagcggcacaaggctcggctcaacctggctaccaggacccggccctacactctcctgttttctcttctcttcatccctgtcttctccaaagcaatgcacgtggcccagcctgctgtggtgctggccaacagccgagggatcgccagctttgtgtgtgagtatgcatctccaggcaaagccactgaggtccgggtgacagtgcttcggcaggccgacagccaggtgactgaagtctgtgcggcaacgtacatgatggggaatgagttgaccttcctagatgattccatctgcacgggcacctccagtggaaatcaagtgaacctcactatccaaggactgagggctatggacacaggactctacatctgcaaggtggagctcatgtacccaccaccatactacatgggcataggcaatggaacccagatttatgtaattgatccagaaccgtgcccagattctgacttcctcctctggatccttgcagcagttagttcggggttgtttttttatagctttctcctcacagctgtttctttgagcaaaatgctaaagaaaagaagccctctcacaacaggggtctatgtgaaaatgcccccaacagagccagaatgtgaaaagcaatttcagccttattttattcccatcaat

SEQ ID NO: 40 - protein, 223 aa, Macaca fascicularis
MACLGFQRHKARLNLATRTRPYTLLFSLLFIPVFSKAMHVAQPAVVLANSRGIASFVCEYASPGKATEVRVTVLRQADSQVTEVCAATYMMGNELTFLDDSICTGTSSGNQVNLTIQGLRAMDTGLYICKVELMYPPPYYMGIGNGTQIYVIDPEPCPDSDFLLWILAAVSSGLFFYSFLLTAVSLSKMLKKRSPLTTGVYVKMPPTEPECEKQFQPYFIPIN

SEQ ID NO: 41 - DNA, 669 bp, Artificial Sequence
  Human-mouse CTLA4
  CDS (1)..(669)
atggcctgcctgggcttccagagacacaaggcccagctgaacctggccaccaggacctggccttgtaccctgctgttcttcctgctgtttatccccgtgttctgcaaggccatgcacgtggcccagcctgctgtggtgctggcctcttccagaggaatcgcctccttcgtgtgcgagtacgcctccccccacaacaccgatgaagtgcgcgtgaccgtgctgcggcagaccaacgaccagatgaccgaagtgtgcgccaccaccttcaccgagaagaacgagctgaccttcctggacgactctatctgcaccggcacctccagcggcaaccaagtgaacctgacaatccagggcctgcgggccatggacaccggcctgtacctgtgcaaggtggaactgatgtacccccctccctacttcgtgggcatgggcaacggcacccagatctacgtgatcgaccccgagccttgccccgactccgactttctgctgtggatcctggctgccgtgtcctccggcctgttcttctactctttcctgctgaccgccgtgtccctgtccaagatgctgaagaagcggtcccccctgaccaccggcgtgggagtgaaaatgcctcccaccgagcccgagtgcgagaagcagttccagcccggcttcatccccatcaac

SEQ ID NO: 42 - protein, 223 aa, Artificial Sequence
  Synthetic Construct
MACLGFQRHKAQLNLATRTWPCTLLFFLLFIPVFCKAMHVAQPAVVLASSRGIASFVCEYASPHNTDEVRVTVLRQTNDQMTEVCATTFTEKNELTFLDDSICTGTSSGNQVNLTIQGLRAMDTGLYLCKVELMYPPPYFVGMGNGTQIYVIDPEPCPDSDFLLWILAAVSSGLFFYSFLLTAVSLSKMLKKRSPLTTGVGVKMPPTEPECEKQFQPGFIPIN

SEQ ID NO: 43 - DNA, 669 bp, Artificial Sequence
  Mouse-Human CTLA4
  CDS (1)..(669)
atggcctgcctgggcttccagagacacaaggcccagctgaacctggccaccaggacctggccttgtaccctgctgttcttcctgctgtttatccccgtgttctgcgaggccatccaagtgacccagccctctgtggtgctggcctcttctcatggcgtggccagcttcccttgcgagtactccccatctggcaaggccaccgaagtgcgcgtgaccgtgctgagacaggccgactcccaagtgacagaagtgtgcgccgccacctacatgatgggcaacaccgtgggctttctggactaccccttctgctccggcaccttcaacgagtccagagtgaacctgacaatccagggcctgcgggccgtggataccggcctgtatatctgcaaggtggaactgatgtacccccctccctactacctgggcatcggcaacggcacccagatctacgtgatcgaccccgagccttgccccgactccgactttctgctgtggatcctggccgccgtgtcctccggcctgttcttctactctttcctgctgaccgctgtgtccctgtccaagatgctgaagaagcggtcccccctgaccaccggcgtgggagtgaaaatgcctcccaccgagcccgagtgcgagaagcagttccagcccggcttcatccccatcaac

SEQ ID NO: 44 - protein, 223 aa, Artificial Sequence
  Synthetic Construct
MACLGFQRHKAQLNLATRTWPCTLLFFLLFIPVFCEAIQVTQPSVVLASSHGVASFPCEYSPSGKATEVRVTVLRQADSQVTEVCAATYMMGNTVGFLDYPFCSGTFNESRVNLTIQGLRAVDTGLYICKVELMYPPPYYLGIGNGTQIYVIDPEPCPDSDFLLWILAAVSSGLFFYSFLLTAVSLSKMLKKRSPLTTGVGVKMPPTEPECEKQFQPGFIPIN

SEQ ID NO: 45 - DNA, 669 bp, Mus musculus
  CDS (1)..(669)
atggcttgtcttggactccggaggtacaaagctcaactgcagctgccttctaggacttggccttttgtagccctgctcactcttcttttcatcccagtcttctctgaagccatacaggtgacccaaccttcagtggtgttggctagcagccatggtgtcgccagctttccatgtgaatattcaccatcacacaacactgatgaggtccgggtgactgtgctgcggcagacaaatgaccaaatgactgaggtctgtgccacgacattcacagagaagaatacagtgggcttcctagattaccccttctgcagtggtacctttaatgaaagcagagtgaacctcaccatccaaggactgagagctgttgacacgggactgtacctctgcaaggtggaactcatgtacccaccgccatactttgtgggcatgggcaacgggacgcagatttatgtcattgatccagaaccatgcccggattctgacttcctcctttggatccttgtcgcagttagcttggggttgtttttttacagtttcctggtctctgctgtttctttgagcaagatgctaaagaaaagaagtcctcttacaacaggggtctatgtgaaaatgcccccaacagagccagaatgtgaaaagcaatttcagccttattttattcccatcaac

SEQ ID NO: 46 - protein, 223 aa, Mus musculus
MACLGLRRYKAQLQLPSRTWPFVALLTLLFIPVFSEAIQVTQPSVVLASSHGVASFPCEYSPSHNTDEVRVTVLRQTNDQMTEVCATTFTEKNTVGFLDYPFCSGTFNESRVNLTIQGLRAVDTGLYLCKVELMYPPPYFVGMGNGTQIYVIDPEPCPDSDFLLWILVAVSLGLFFYSFLVSAVSLSKMLKKRSPLTTGVYVKMPPTEPECEKQFQPYFIPIN

SEQ ID NO: 47 - DNA, 990 bp, Artificial Sequence
  human IgG1 constant domains
  CDS (1)..(990)
gccagcacaaagggcccatcggtcttccccctggcaccctcctccaagagcacctctgggggcacagcggccctgggctgcctggtcaaggactacttccccgaaccggtgacggtgtcgtggaactcaggcgccctgaccagcggcgtgcacaccttcccggctgtcctacagtcctcaggactctactccctcagcagcgtggtgaccgtgccctccagcagcttgggcacccagacctacatctgcaacgtgaatcacaagcccagcaacaccaaggtggacaagaaagttgagcccaaatcttgtgacaaaactcacacatgcccaccgtgcccagcacctgaactcctggggggaccgtcagtcttcctcttccccccaaaacccaaggacaccctcatgatctcccggacccctgaggtcacatgcgtggtggtggacgtgagccacgaagaccctgaggtcaagttcaactggtacgtggacggcgtggaggtgcataatgccaagacaaagccgcgggaggagcagtacaacagcacgtaccgggtggtcagcgtcctcaccgtcctgcaccaggactggctgaatggcaaggagtacaagtgcaaggtctccaacaaagccctcccagcccccatcgagaaaaccatctccaaagccaaagggcagccccgagaaccacaggtgtacaccctgcccccatcccgggatgagctgaccaagaaccaggtcagcctgacctgcctggtcaaaggcttctatcccagcgacatcgccgtggagtgggagagcaatgggcagccggagaacaactacaagaccacgcctcccgtgctggactccgacggctccttcttcctctacagcaagctcaccgtggacaagagcaggtggcagcaggggaacgtcttctcatgctccgtgatgcatgaggctctgcacaaccactacacgcagaagagcctctccctgtctccgggtaaa

SEQ ID NO: 48 - protein, 330 aa, Artificial Sequence [sequence omitted]

SEQ ID NO: 49 - DNA, 981 bp, Artificial Sequence
  human IgG4 constant domains (including S228P)
  CDS (1)..(981)
gccagcacaaagggccccagcgtgttccctctggccccttgtagcagaagcaccagcgagtctacagccgccctgggctgcctcgtgaaggactactttcccgagcccgtgaccgtgtcctggaactctggcgctctgacaagcggcgtgcacacctttccagccgtgctgcagagcagcggcctgtactctctgagcagcgtcgtgactgtgcccagcagctctctgggcaccaagacctacacctgtaacgtggaccacaagcccagcaacaccaaggtggacaagcgggtggaatctaagtacggccctccctgccctccttgcccagcccctgaatttctgggcggaccctccgtgttcctgttccccccaaagcccaaggacaccctgatgatcagccggacccccgaagtgacctgcgtggtggtggatgtgtcccaggaagatcctgaggtgcagttcaattggtacgtggacggcgtggaagtgcacaacgccaagaccaagcctagagaggaacagttcaacagcacctaccgggtggtgtccgtgctgacagtgctgcaccaggactggctgaacggcaaagagtacaagtgcaaggtgtccaacaagggactgcccagctccatcgagaaaaccatcagcaaggccaagggccagccccgcgaaccccaggtgtacacactgcctccaagccaggaagagatgaccaagaaccaggtgtccctgacctgtctcgtgaaaggcttctacccctccgatatcgccgtggaatgggagagcaacggccagcccgagaacaactacaagaccaccccccctgtgctggacagcgacggctcattcttcctgtacagcagactgaccgtggacaagagccggtggcaggaaggcaacgtgttcagctgcagcgtgatgcacgaggccctgcacaaccactacacccagaagtccctgtctctgagcctgggcaaa

SEQ ID NO: 50 - protein, 327 aa, Artificial Sequence
  Synthetic Construct
ASTKGPSVFPLAPCSRSTSESTAALGCLVKDYFPEPVTVSWNSGALTSGVHTFPAVLQSSGLYSLSSVVTVPSSSLGTKTYTCNVDHKPSNTKVDKRVESKYGPPCPPCPAPEFLGGPSVFLFPPKPKDTLMISRTPEVTCVVVDVSQEDPEVQFNWYVDGVEVHNAKTKPREEQFNSTYRVVSVLTVLHQDWLNGKEYKCKVSNKGLPSSIEKTISKAKGQPREPQVYTLPPSQEEMTKNQVSLTCLVKGFYPSDIAVEWESNGQPENNYKTTPPVLDSDGSFFLYSRLTVDKSRWQEGNVFSCSVMHEALHNHYTQKSLSLSLGK

SEQ ID NO: 51 - DNA, 321 bp, Artificial Sequence
  human kappa constant domain
  CDS (1)..(321)
cggacagtggccgctcccagcgtgttcatcttcccacctagcgacgagcagctgaagtccggcacagcctctgtcgtgtgcctgctgaacaacttctacccccgcgaggccaaggtgcagtggaaggtggacaatgccctgcagagcggcaacagccaggaaagcgtgaccgagcaggacagcaaggactccacctacagcctgagcagcaccctgacactgagcaaggccgactacgagaagcacaaggtgtacgcctgcgaagtgacccaccagggcctgtctagccccgtgaccaagagcttcaaccggggcgagtgc

SEQ ID NO: 52 - protein, 107 aa, Artificial Sequence [sequence omitted]

SEQ ID NO: 53 - protein, 13 aa, Homo sapiens
SFVCEYASPGKAT

SEQ ID NO: 54 - protein, 25 aa, Homo sapiens
VLASSRGIASFVCEYASPGKATEVR

SEQ ID NO: 55 - protein, 9 aa, Homo sapiens
ASSRGIASF

SEQ ID NO: 56 - protein, 5 aa, Homo sapiens
ATEVR

SEQ ID NO: 57 - protein, 8 aa, Homo sapiens
ASPGKATE

SEQ ID NO: 58 - protein, 31 aa, Homo sapiens
VLASSRGIASFVCEYASPGKATEVRVTVLRQ

SEQ ID NO: 59 - protein, 369 aa, Artificial Sequence
  rhCTLA-4/Fc/6His
AMHVAQPAVVLASSRGIASFVCEYASPGKATEVRVTVLRQADSQVTEVCAATYMMGNELTFLDDSICTGTSSGNQVNLTIQGLRAMDTGLYICKVELMYPPPYYLGIGNGTQIYVIDPEPCPDSDFIEGRMDPKSCDKTHTCPPCPAPELLGGPSVFLFPPKPKDTLMISRTPEVTCVVVDVSHEDPEVKFNWYVDGVEVHNAKTKPREEQYNSTYRVVSVLTVLHQDWLNGKEYKCKVSNKALPAPIEKTISKAKGQPREPQVYTLPPSRDELTKNQVSLTCLVKGFYPSDIAVEWESNGQPENNYKTTPPVLDSDGSFFLYSKLTVDKSRWQQGNVFSCSVMHEALHNHYTQKSLSLSPGKHHHHHH